European Patent Application EP 4 591 877 A1, published July 30, 2025. Title: BCMA 특이적 키메라 항원 수용체를 포함하는 신규한 골수 침윤 림프구 집단 및 이의 제조방법. Applicant: 주식회사 박셀바이오. Application KR. The sequence listing filed with the application follows.

SEQUENCE LISTING (13 sequences)

SEQ ID NO: 1 - protein, 492 aa, synthetic construct
QVQLQESGGGSVQPGGSLRLSCKASGFTFSPSAMSWARQAPGKEIEWVSNIYPDGRTYYADSMKGRFTISRDNAENTVYLQMNSLKPEDTAVYYCLIGVGIVAGQVVSPYWGQGTQVTVSSGGGGSGGGGSGGGGSGGGGSGGGGSQVQLQESGGGLVQPGGSLRLSCAASGFTFSNYAMSWFRQGPGKERELVAGIDRTGGSTRTADSVQGRFTISRDNAKNKVYLQMNSLKPEDTAVYYCKALRTPGWGTSPDVVGYWGQGTQVTVSSTTPAPRPPTPAPTIASQPLSLRPEACRPAAGGAVHTRGLDFACDIYIWAPLAGTCGVLLLSLVITLYCKRGRKKLLYIFKQPFMRPVQTTQEEDGCSCRFPEEEEGGCELRVKFSRSADAPAYKQGQNQLYNELNLGRREEYDVLDKRRGRDPEMGGKPRRKNPQEGLYNELQKDKMAEAYSEIGMKGERRRGKGHDGLYQGLSTATKDTYDALHMQALPPR

SEQ ID NO: 2 - protein, 8 aa, synthetic construct
GFTFSPSA

SEQ ID NO: 3 - protein, 8 aa, synthetic construct
GFTFSNYA

SEQ ID NO: 4 - protein, 7 aa, synthetic construct
IYPDGRT

SEQ ID NO: 5 - protein, 8 aa, synthetic construct
IDRTGGST

SEQ ID NO: 6 - protein, 15 aa, synthetic construct
LIGVGIVAGQVVSPY

SEQ ID NO: 7 - protein, 17 aa, synthetic construct
KALRTPGWGTSPDVVGY

SEQ ID NO: 8 - protein, 121 aa, synthetic construct
QVQLQESGGGSVQPGGSLRLSCKASGFTFSPSAMSWARQAPGKEIEWVSNIYPDGRTYYADSMKGRFTISRDNAENTVYLQMNSLKPEDTAVYYCLIGVGIVAGQVVSPYWGQGTQVTVSS

SEQ ID NO: 9 - protein, 124 aa, synthetic construct
QVQLQESGGGLVQPGGSLRLSCAASGFTFSNYAMSWFRQGPGKERELVAGIDRTGGSTRTADSVQGRFTISRDNAKNKVYLQMNSLKPEDTAVYYCKALRTPGWGTSPDVVGYWGQGTQVTVSS

SEQ ID NO: 10 - protein, 70 aa, synthetic construct
TTPAPRPPTPAPTIASQPLSLRPEACRPAAGGAVHTRGLDFACDIYIWAPLAGTCGVLLLSLVITLYCKR

SEQ ID NO: 11 - protein, 42 aa, synthetic construct
GRKKLLYIFKQPFMRPVQTTQEEDGCSCRFPEEEEGGCELRV

SEQ ID NO: 12 - protein, 110 aa, synthetic construct
KFSRSADAPAYKQGQNQLYNELNLGRREEYDVLDKRRGRDPEMGGKPRRKNPQEGLYNELQKDKMAEAYSEIGMKGERRRGKGHDGLYQGLSTATKDTYDALHMQALPPR

SEQ ID NO: 13 - DNA, 2721 bp, synthetic construct
  source 1..2721: mol_type = other DNA
ggctccggtgcccgtcagtgggcagagcgcacatcgcccacagtccccgagaagttggggggaggggtcggcaattgaaccggtgcctagagaaggtggcgcggggtaaactgggaaagtgatgtcgtgtactggctccgcctttttcccgagggtgggggagaaccgtatataagtgcagtagtcgccgtgaacgttctttttcgcaacgggtttgccgccagaacacaggtaagtgccgtgtgtggttcccgcgggcctggcctctttacgggttatggcccttgcgtgccttgaattacttccacctggctgcagtacgtgattcttgatcccgagcttcgggttggaagtgggtgggagagttcgaggccttgcgcttaaggagccccttcgcctcgtgcttgagttgaggcctggcctgggcgctggggccgccgcgtgcgaatctggtggcaccttcgcgcctgtctcgctgctttcgataagtctctagccatttaaaatttttgatgacctgctgcgacgctttttttctggcaagatagtcttgtaaatgcgggccaagatctgcacactggtatttcggtttttggggccgcgggcggcgacggggcccgtgcgtcccagcgcacatgttcggcgaggcggggcctgcgagcgcggccaccgagaatcggacgggggtagtctcaagctggccggcctgctctggtgcctggcctcgcgccgccgtgtatcgccccgccctgggcggcaaggctggcccggtcggcaccagttgcgtgagcggaaagatggccgcttcccggccctgctgcagggagctcaaaatggaggacgcggcgctcgggagagcgggcgggtgagtcacccacacaaaggaaaagggcctttccgtcctcagccgtcgcttcatgtgactccacggagtaccgggcgccgtccaggcacctcgattagttctcgagcttttggagtacgtcgtctttaggttggggggaggggttttatgcgatggagtttccccacactgagtgggtggagactgaagttaggccagcttggcacttgatgtaattctccttggaatttgccctttttgagtttggatcttggttcattctcaagcctcagacagtggttcaaagtttttttcttccatttcaggtgtcgtgaatgctgctgctggtgaccagcctgctgctgtgcgagctgccccaccccgcctttctgctgatcccccaggtgcagctgcaggagtctggaggaggctcggtacagcctggggggtctctgagactctcctgtaaagcctctggattcaccttcagtccctctgccatgagctgggcccgccaggcaccagggaaggagatcgagtgggtgtccaatatttaccctgatggacgcacatactatgcggactccatgaagggccgattcaccatctccagagacaacgccgagaacacggtgtatctgcaaatgaacagcctgaaacctgaggacacggccgtttattactgtctaataggagtcggtattgtggccggtcaggtagtttcgccctactggggtcaggggacccaggtcaccgtctcctcaggaggcggaggatctggcggaggtggaagtggcggaggcggttctggtggtggtggctctggtggcggcggatctcaggtgcagctgcaggagtctggaggaggcttggtgcagcctggggggtctctgagactctcctgtgcagcctctggattcaccttcagtaactatgccatgagctggttccgccagggtccagggaaggagcgcgagttggtcgcaggtatcgatcgtactggaggtagcacaaggactgcagactccgtgcagggccgattcaccatctccagagacaatgccaagaacaaggtgtatctgcaaatgaatagcctgaaacctgaggacacggccgtgtattattgtaaggcactgaggactccgggctggggtacgtctcccgatgtcgttggctactggggccaggggacccaggtcaccgtctcctcaactaccccagcaccgcggccgcccaccccggctcctaccatcgcctcccagcctctgtccctgcgtccggaggcatgtagacccgcagctggtggggccgtgcatacccggggtcttgacttcgcctgcgatatctacatttgggcccctctggctggtacttgcggggtcctgctgctttcactcgtgatcactctttactgtaagcgcggtcggaagaagctgctgtacatctttaagcaacccttcatgaggcctgtgcagactactcaagaggaggacggctgttcatgccggttcccagaggaggaggaaggcggctgcgaactgcgcgtgaaattcagccgcagcgcagatgctccagcctacaagcaggggcagaaccagctctacaacgaactcaatcttggtcggagagaggagtacgacgtgctggacaagcggagaggacgggacccagaaatgggcgggaagccgcgcagaaagaatccccaagagggcctgtacaacgagctccaaaaggataagatggcagaagcctatagcgagattggtatgaaaggggaacgcagaagaggcaaaggccacgacggactgtaccagggactcagcaccgccaccaaggacacctatgacgctcttcacatgcaggccctgccgcctcgg